European Patent Specification EP 3 626 274 B1, published January 22, 2025. Title: RECOMBINANT PROMOTERS AND VECTORS FOR PROTEIN EXPRESSION IN LIVER AND USE THEREOF. Applicant: Emory University CHILDREN'S HEALTHCARE OF ATLANTA, INC. Doering, Christopher Spencer, H Trent Brown, Harrison C. The sequence listing filed with the application follows.

SEQUENCE LISTING (131 sequences)

SEQ ID NO: 1 - protein, 2351 aa, homo sapiens
MQIELSTCFFLCLLRFCFSATRRYYLGAVELSWDYMQSDLGELPVDARFPPRVPKSFPFNTSVVYKKTLFVEFTDHLFNIAKPRPPWMGLLGPTIQAEVYDTVVITLKNMASHPVSLHAVGVSYWKASEGAEYDDQTSQREKEDDKVFPGGSHTYVWQVLKENGPMASDPLCLTYSYLSHVDLVKDLNSGLIGALLVCREGSLAKEKTQTLHKFILLFAVFDEGKSWHSETKNSLMQDRDAASARAWPKMHTVNGYVNRSLPGLIGCHRKSVYWHVIGMGTTPEVHSIFLEGHTFLVRNHRQASLEISPITFLTAQTLLMDLGQFLLFCHISSHQHDGMEAYVKVDSCPEEPQLRMKNNEEAEDYDDDLTDSEMDVVRFDDDNSPSFIQIRSVAKKHPKTWVHYIAAEEEDWDYAPLVLAPDDRSYKSQYLNNGPQRIGRKYKKVRFMAYTDETFKTREAIQHESGILGPLLYGEVGDTLLIIFKNQASRPYNIYPHGITDVRPLYSRRLPKGVKHLKDFPILPGEIFKYKWTVTVEDGPTKSDPRCLTRYYSSFVNMERDLASGLIGPLLICYKESVDQRGNQIMSDKRNVILFSVFDENRSWYLTENIQRFLPNPAGVQLEDPEFQASNIMHSINGYVFDSLQLSVCLHEVAYWYILSIGAQTDFLSVFFSGYTFKHKMVYEDTLTLFPFSGETVFMSMENPGLWILGCHNSDFRNRGMTALLKVSSCDKNTGDYYEDSYEDISAYLLSKNNAIEPRSFSQNSRHPSTRQKQFNATTIPENDIEKTDPWFAHRTPMPKIQNVSSSDLLMLLRQSPTPHGLSLSDLQEAKYETFSDDPSPGAIDSNNSLSEMTHFRPQLHHSGDMVFTPESGLQLRLNEKLGTTAATELKKLDFKVSSTSNNLISTIPSDNLAAGTDNTSSLGPPSMPVHYDSQLDTTLFGKKSSPLTESGGPLSLSEENNDSKLLESGLMNSQESSWGKNVSSTESGRLFKGKRAHGPALLTKDNALFKVSISLLKTNKTSNNSATNRKTHIDGPSLLIENSPSVWQNILESDTEFKKVTPLIHDRMLMDKNATALRLNHMSNKTTSSKNMEMVQQKKEGPIPPDAQNPDMSFFKMLFLPESARWIQRTHGKNSLNSGQGPSPKQLVSLGPEKSVEGQNFLSEKNKVVVGKGEFTKDVGLKEMVFPSSRNLFLTNLDNLHENNTHNQEKKIQEEIEKKETLIQENVVLPQIHTVTGTKNFMKNLFLLSTRQNVEGSYDGAYAPVLQDFRSLNDSTNRTKKHTAHFSKKGEEENLEGLGNQTKQIVEKYACTTRISPNTSQQNFVTQRSKRALKQFRLPLEETELEKRIIVDDTSTQWSKNMKHLTPSTLTQIDYNEKEKGAITQSPLSDCLTRSHSIPQANRSPLPIAKVSSFPSIRPIYLTRVLFQDNSSHLPAASYRKKDSGVQESSHFLQGAKKNNLSLAILTLEMTGDQREVGSLGTSATNSVTYKKVENTVLPKPDLPKTSGKVELLPKVHIYQKDLFPTETSNGSPGHLDLVEGSLLQGTEGAIKWNEANRPGKVPFLRVATESSAKTPSKLLDPLAWDNHYGTQIPKEEWKSQEKSPEKTAFKKKDTILSLNACESNHAIAAINEGQNKPEIEVTWAKQGRTERLCSQNPPVLKRHQREITRTTLQSDQEEIDYDDTISVEMKKEDFDIYDEDENQSPRSFQKKTRHYFIAAVERLWDYGMSSSPHVLRNRAQSGSVPQFKKVVFQEFTDGSFTQPLYRGELNEHLGLLGPYIRAEVEDNIMVTFRNQASRPYSFYSSLISYEEDQRQGAEPRKNFVKPNETKTYFWKVQHHMAPTKDEFDCKAWAYFSDVDLEKDVHSGLIGPLLVCHTNTLNPAHGRQVTVQEFALFFTIFDETKSWYFTENMERNCRAPCNIQMEDPTFKENYRFHAINGYIMDTLPGLVMAQDQRIRWYLLSMGSNENIHSIHFSGHVFTVRKKEEYKMALYNLYPGVFETVEMLPSKAGIWRVECLIGEHLHAGMSTLFLVYSNKCQTPLGMASGHIRDFQITASGQYGQWAPKLARLHYSGSINAWSTKEPFSWIKVDLLAPMIIHGIKTQGARQKFSSLYISQFIIMYSLDGKKWQTYRGNSTGTLMVFFGNVDSSGIKHNIFNPPIIARYIRLHPTHYSIRSTLRMELMGCDLNSCSMPLGMESKAISDAQITASSYFTNMFATWSPSKARLHLQGRSNAWRPQVNNPKEWLQVDFQKTMKVTGVTTQGVKSLLTSMYVKEFLISSSQDGHQWTLFFQNGKVKVFQGNQDSFTPVVNSLDPPLLTRYLRIHPQSWVHQIALRMEVLGCEAQDLY

SEQ ID NO: 2 - DNA, 4374 bp, Artificial Sequence
  recombinant fVIII
atgcagattgaactgtctacctgtttctttctgtgcctgctgaggttttgtttttctgctaccagaagatactacctgggagctgtggaactgagctgggattacatgcagtctgacctgggagagctgcctgtggatgctagattcccacctagagtccctaagtccttccccttcaacacctctgtggtctacaagaaaaccctgtttgtggagtttacagaccacctgttcaacattgctaagcctagaccaccatggatgggactgctgggaccaaccatccaggcagaggtgtatgacacagtggtcatcaccctgaaaaacatggcttctcaccctgtgtccctgcatgctgtgggagtctcctactggaaggcctctgaaggggctgagtatgatgatcagaccagccagagggaaaaagaggatgataaggtgttccctggagggtcccatacctatgtgtggcaggtcctgaaggagaatggaccaatggcttctgaccctctgtgcctgacctactcttatctgtcccatgtggacctggtcaaggatctgaactctggcctgattggggctctgctggtgtgtagggaagggtccctggccaaggagaaaacccagaccctgcataagttcatcctgctgtttgctgtgtttgatgaaggaaaaagctggcactctgagaccaagaactctctgatgcaggacagggatgctgcttctgccagagcttggcccaagatgcacacagtgaatggctatgtcaataggagcctgcctggactgattggctgccacagaaagtctgtgtattggcatgtcattggaatgggcaccacccctgaagtgcacagcatcttcctggaggggcatacctttctggtcaggaaccacaggcaggctagcctggagatctctccaatcaccttcctgacagcccagaccctgctgatggacctgggacagttcctgctgttttgccacatctccagccaccagcatgatggcatggaggcttatgtgaaagtggactcctgtcctgaggaacctcagctgaggatgaagaacaatgaggaagctgaagactatgatgatgacctgacagactctgagatggatgtggtcaggtttgatgatgataactctccctcctttatccagatcaggtctgtggccaagaaacaccctaagacctgggtccattacattgctgctgaggaagaggactgggattatgctccactggtgctggcccctgatgatagatcctacaaaagccagtatctgaacaatggaccccagaggattggcagaaagtacaagaaagtgaggttcatggcttatacagatgagacctttaagaccagagaagccatccagcatgagtctgggatcctgggacctctgctgtatggggaagtgggggacaccctgctgatcatcttcaagaaccaggccagcaggccttacaatatctatccacatggcatcacagatgtgagacctctgtactccaggaggctgccaaagggggtgaaacacctgaaggacttcccaatcctgcctggggaaatctttaagtataaatggacagtcacagtggaggatgggcccaccaagtctgaccctaggtgcctgaccagatactattcttcctttgtgaatatggagagagacctggcttctggactgattggacccctgctgatctgttacaaagagtctgtggatcagaggggcaaccagatcatgtctgacaagaggaatgtgatcctgttctctgtctttgatgaaaacaggtcttggtacctgacagagaacatccagaggttcctgcctaatccagctggagtgcagctggaagatcctgagttccaggcctctaacatcatgcattccatcaatggctatgtgtttgactccctgcagctgtctgtgtgcctgcatgaggtggcttactggtatatcctgagcattggagcccagacagatttcctgtctgtgttcttttctggctacacctttaagcataaaatggtgtatgaggacaccctgaccctgttcccattttctggagaaactgtgttcatgagcatggagaatcctgggctgtggatcctgggatgccacaactctgatttcaggaatagagggatgacagccctgctgaaagtgagctcttgtgacaagaacacaggagactactatgaagatagctatgaggacatctctgcttatctgctgtccaaaaacaatgccattgagcccaggagcttctctcagaaccctccagtgctgaagaggcaccagagggagatcaccagaaccaccctgcagtctgatcaggaagagattgactatgatgataccatctctgtggaaatgaagaaagaggactttgatatctatgatgaagatgagaaccagtctcccaggtccttccagaagaaaaccagacattactttattgctgctgtggagaggctgtgggactatggcatgtccagctctcctcatgtgctgagaaatagagctcagtctggatctgtcccacagttcaagaaagtggtcttccaggagtttacagatggaagctttacccagccactgtacaggggagaactgaatgagcacctggggctgctgggaccctatatcagggctgaagtggaggataacatcatggtcaccttcaggaatcaggccagcagaccctactctttttattccagcctgatctcctatgaagaggaccagagacagggagctgaaccaagaaaaaactttgtgaagcctaatgagaccaaaacctacttttggaaggtgcagcaccatatggcccctaccaaagatgagtttgattgcaaggcctgggcttatttttctgatgtggatctggagaaggatgtccactctggcctgattgggccactgctggtgtgtcataccaacaccctgaatccagctcatggaaggcaggtgacagtccaggaatttgccctgttctttaccatctttgatgagaccaagagctggtacttcacagaaaacatggagaggaattgcagagccccatgtaacatccagatggaagaccccaccttcaaggagaactacagatttcatgctatcaatgggtatatcatggataccctgccaggactggtcatggctcaggaccagaggatcagatggtacctgctgagcatggggtctaatgagaatatccactccatccatttctctggacatgtgtttacagtaaggaagaaagaagagtacaagatggccctgtacaacctgtatcctggggtgtttgaaacagtggagatgctgccttccaaggctgggatctggagggtggaatgcctgattggggagcacctgcatgctggaatgtctaccctgttcctggtgtactccaataagtgtcagacccccctggggatggcttctggacatatcagggacttccagatcacagcttctggacagtatggacagtgggctcctaagctggctagactgcactattctggctccatcaatgcttggtctaccaaagagcctttctcctggatcaaggtggacctgctggctccaatgatcatccatggcatcaaaacccagggggccaggcagaagttctcttccctgtacatcagccagtttatcatcatgtattctctggatgggaagaaatggcagacctacagaggcaattccacagggaccctgatggtgttctttggcaatgtggacagctctgggatcaagcacaacatcttcaatccccctatcattgccaggtacatcagactgcacccaacccattattccatcaggagcaccctgagaatggagctgatggggtgtgatctgaacagctgttctatgcccctgggaatggagtctaaggccatctctgatgctcagatcacagcctccagctacttcaccaatatgtttgctacctggtccccaagcaaggctagactgcatctgcagggaagaagcaatgcttggagaccacaggtgaacaatcccaaggagtggctgcaggtggacttccagaaaaccatgaaggtgacaggagtcaccacccagggagtgaaaagcctgctgacctctatgtatgtcaaggagttcctgatctcttccagccaggatgggcaccagtggaccctgttctttcagaatggaaaggtgaaagtcttccagggcaatcaggattcctttacccctgtggtcaacagcctggacccacccctgctgaccaggtacctgagaatccacccacagtcctgggtgcatcagattgctctgaggatggaagtcctgggctgtgaggcccaggacctgtattga

SEQ ID NO: 3 - protein, 1457 aa, Artificial Sequence
  recombinant fVIII
MQIELSTCFFLCLLRFCFSATRRYYLGAVELSWDYMQSDLGELPVDARFPPRVPKSFPFNTSVVYKKTLFVEFTVHLFNIAKPRPPWMGLLGPTIQAEVYDTVVITLKNMASHPVSLHAVGVSYWKASEGAEYDDQTSQREKEDDKVFPGGSHTYVWQVLKENGPMASDPLCLTYSYLSHVDLVKDLNSGLIGALLVCREGSLAKEKTQTLHKFILLFAVFDEGKSWHSETKNSLMQDRDAASARAWPKMHTVNGYVNRSLPGLIGCHRKSVYWHVIGMGTTPEVHSIFLEGHTFLVRNHRQASLEISPITFLTAQTLLMDLGQFLLFCHISSHQHDGMEAYVKVDSCPEEPQLRMKNNEEAEDYDDDLTDSEMDVVRFDDDNSPSFIQIRSVAKKHPKTWVHYIAAEEEDWDYAPLVLAPDDRSYKSQYLNNGPQRIGRKYKKVRFMAYTDETFKTREAIQHESGILGPLLYGEVGDTLLIIFKNQASRPYNIYPHGITDVRPLYSRRLPKGVKHLKDFPILPGEIFKYKWTVTVEDGPTKSDPRCLTRYYSSFVNMERDLASGLIGPLLICYKESVDQRGNQIMSDKRNVILFSVFDENRSWYLTENIQRFLPNPAGVQLEDPEFQASNIMHSINGYVFDSLQLSVCLHEVAYWYILSIGAQTDFLSVFFSGYTFKHKMVYEDTLTLFPFSGETVFMSMENPGLWILGCHNSDFRNRGMTALLKVSSCDKNTGDYYEDSYEDISAYLLSKNNAIEPRSFSQNPPVLKRHQREITRTTLQSDQEEIDYDDTISVEMKKEDFDIYDEDENQSPRSFQKKTRHYFIAAVERLWDYGMSSSPHVLRNRAQSGSVPQFKKVVFQEFTDGSFTQPLYRGELNEHLGLLGPYIRAEVEDNIMVTFRNQASRPYSFYSSLISYEEDQRQGAEPRKNFVKPNETKTYFWKVQHHMAPTKDEFDCKAWAYFSDVDLEKDVHSGLIGPLLVCHTNTLNPAHGRQVTVQEFALFFTIFDETKSWYFTENMERNCRAPCNIQMEDPTFKENYRFHAINGYIMDTLPGLVMAQDQRIRWYLLSMGSNENIHSIHFSGHVFTVRKKEEYKMALYNLYPGVFETVEMLPSKAGIWRVECLIGEHLHAGMSTLFLVYSNKCQTPLGMASGHIRDFQITASGQYGQWAPKLARLHYSGSINAWSTKEPFSWIKVDLLAPMIIHGIKTQGARQKFSSLYISQFIIMYSLDGKKWQTYRGNSTGTLMVFFGNVDSSGIKHNIFNPPIIARYIRLHPTHYSIRSTLRMELMGCDLNSCSMPLGMESKAISDAQITASSYFTNMFATWSPSKARLHLQGRSNAWRPQVNNPKEWLQVDFQKTMKVTGVTTQGVKSLLTSMYVKEFLISSSQDGHQWTLFFQNGKVKVFQGNQDSFTPVVNSLDPPLLTRYLRIHPQSWVHQIALRMEVLGCEAQDLY

SEQ ID NO: 4 - DNA, 146 bp, Artificial Sequence
  recombinant promoter sequence
gttaatcattaagtcgttaatttttgtggcccttgcgatgtttgctctggttaataatctcaggacaaacagaggttaataattttccagatctctctgagcaatagtataaaaggccagcagcagcctgaccacatctcatcctc

SEQ ID NO: 5 - DNA, 159 bp, Artificial Sequence
  recombinant promoter sequence
gttaatttttgtggcccttgcgatgtttgctctggttaataatctcaggacaaacatacattttcagtcatatgtttgctcactgaaggttactagttaacaggcatcccttaaacaggatataaaaggccagcagcagcctgaccacatctcatcctc

SEQ ID NO: 6 - DNA, 172 bp, Artificial Sequence
  recombinant promoter sequence
gttaatttttaaaaagcagtcaaaagtccaagtggcccttgcgagcatttactctctctgtttgctctggttaataatctcaggagcacaaacagaggttaataattttcagtcatatgtttgctcactgaaggttactagttaacaggcatcccttaaacaggatataaaa

SEQ ID NO: 7 - DNA, 204 bp, Artificial Sequence
  recombinant promoter sequence
gttaatttttaaaaagcagtcaaaagtccaagtggcccttgcgagcatttactctctctgtttgctctggttaataatctcaggagcacaaacagaggttaataattttcagtcatatgtttgctcactgaaggttactagttaacaggcatcccttaaacaggatataaaaggccagcagcagcctgaccacatctcatcctc

SEQ ID NO: 8 - DNA, 1386 bp, Artificial Sequence
  recombinant fIX
atgcagagggtgaacatgatcatggctgagtctcctggactgatcaccatctgcctgctgggctatctgctgtctgctgagtgtacagtgttcctggaccatgaaaatgctaataaaatcctgaacaggccaaagaggtacaattctgggaaactggaggaatttgtgcagggaaacctggagagggaatgcatggaggaaaagtgtagctttgaggaagccagggaggtgtttgaaaatacagagaggaccacagagttctggaaacagtatgtggatggggatcagtgtgagtccaacccctgtctgaatggagggtcttgcaaggatgatatcaactcctatgagtgctggtgtccttttggatttgaaggcaagaattgtgagctggatgtgacctgtaacatcaaaaatgggaggtgtgagcagttctgtaagaactctgctgataataaagtggtctgcagctgtacagaaggctacaggctggctgagaaccagaagagctgtgaaccagctgtgcccttcccttgtgggagggtgtctgtcagccagaccagcaagctgaccagagctgaggctgtgtttcctgatgtggattatgtcaactctacagaggctgaaaccatcctggacaacatcacccagtctacccagtccttcaatgactttaccagggtggtgggaggggaggatgctaagccaggacagttcccctggcaggtggtcctgaatggcaaagtggatgctttttgtgggggctccattgtgaatgagaagtggattgtcacagctgctcactgtgtggaaactggggtcaagatcacagtggtggctggagagcacaacattgaggaaactgaacatacagagcagaaaaggaatgtgatcagaatcatcccccaccataactacaatgctgctatcaacaagtataatcatgacattgccctgctggaactggatgagcctctggtgctgaacagctatgtcaccccaatctgcattgctgacaaggagtataccaatatcttcctgaaatttgggtctggatatgtgtctgggtggggaagggtcttccacaagggaaggtctgctctggtgctgcagtatctgagggtgcccctggtggacagagctacctgcctgaggagcaccaagttcaccatctacaacaatatgttctgtgctggatttcatgagggagggagggactcctgtcagggagattctggaggccctcatgtgacagaggtggaaggcaccagcttcctgactggcatcatctcttggggggaggaatgtgctatgaaggggaaatatggaatctataccaaggtgtccagatatgtcaactggatcaaggagaaaaccaagctgacctga

SEQ ID NO: 9 - DNA, 1386 bp, Artificial Sequence
  recombinant fIX
atgcagagggtgaacatgatcatggctgagtctcctggactgatcaccatctgcctgctgggctatctgctgtctgctgagtgtacagtgttcctggaccatgaaaatgctaataaaatcctgaacaggccaaagaggtacaattctgggaaactggaggaatttgtgcagggaaacctggagagggaatgcatggaggaaaagtgtagctttgaggaagccagggaggtgtttgaaaatacagagaggaccacagagttctggaaacagtatgtggatggggatcagtgtgagtccaacccctgtctgaatggagggtcttgcaaggatgatatcaactcctatgagtgctggtgtccttttggatttgaaggcaagaattgtgagctggatgtgacctgtaacatcaaaaatgggaggtgtgagcagttctgtaagaactctgctgataataaagtggtctgcagctgtacagaaggctacaggctggctgagaaccagaagagctgtgaaccagctgtgcccttcccttgtgggagggtgtctgtcagccagaccagcaagctgaccagagctgaggctgtgtttcctgatgtggattatgtcaactctacagaggctgaaaccatcctggacaacatcacccagtctacccagtccttcaatgactttaccagggtggtgggaggggaggatgctaagccaggacagttcccctggcaggtggtcctgaatggcaaagtggatgctttttgtgggggctccattgtgaatgagaagtggattgtcacagctgctcactgtgtggaaactggggtcaagatcacagtggtggctggagagcacaacattgaggaaactgaacatacagagcagaaaaggaatgtgatcagaatcatcccccaccataactacaatgctgctatcaacaagtataatcatgacattgccctgctggaactggatgagcctctggtgctgaacagctatgtcaccccaatctgcattgctgacaaggagtataccaatatcttcctgaaatttgggtctggatatgtgtctgggtggggaagggtcttccacaagggaaggtctgctctggtgctgcagtatctgagggtgcccctggtggacagagctacctgcctgctgagcaccaagttcaccatctacaacaatatgttctgtgctggatttcatgagggagggagggactcctgtcagggagattctggaggccctcatgtgacagaggtggaaggcaccagcttcctgactggcatcatctcttggggggaggaatgtgctatgaaggggaaatatggaatctataccaaggtgtccagatatgtcaactggatcaaggagaaaaccaagctgacctga

SEQ ID NO: 10 - DNA, 1386 bp, Artificial Sequence
  recombinant fIX
atgcagagggtgaacatgatcatggctgagtctcctggactgatcaccatctgcctgctgggctatctgctgtctgctgagtgtacagtgttcctggaccatgaaaatgctaataaaatcctgaacaggccaaagaggtacaattctgggaaactggaggaatttgtgcagggaaacctggagagggaatgcatggaggaaaagtgtagctttgaggaagccagggaggtgtttgaaaatacagagaggaccacagagttctggaaacagtatgtggatggggatcagtgtgagtccaacccctgtctgaatggagggtcttgcaaggatgatatcaactcctatgagtgctggtgtccttttggatttgaaggcaagaattgtgagctggatgtgacctgtaacatcaaaaatgggaggtgtgagcagttctgtaagaactctgctgataataaagtggtctgcagctgtacagaaggctacaggctggctgagaaccagaagagctgtgaaccagctgtgcccttcccttgtgggagggtgtctgtcagccagaccagcaagctgaccagagctgagacagtgtttcctgatgtggattatgtcaactctacagaggctgaaaccatcctggacaacatcacccagtctacccagtccttcaatgactttaccagggtggtgggaggggaggatgctaagccaggacagttcccctggcaggtggtcctgaatggcaaagtggatgctttttgtgggggctccattgtgaatgagaagtggattgtcacagctgctcactgtgtggaaactggggtcaagatcacagtggtggctggagagcacaacattgaggaaactgaacatacagagcagaaaaggaatgtgatcagaatcatcccccaccataactacaatgctgctatcaacaagtataatcatgacattgccctgctggaactggatgagcctctggtgctgaacagctatgtcaccccaatctgcattgctgacaaggagtataccaatatcttcctgaaatttgggtctggatatgtgtctgggtggggaagggtcttccacaagggaaggtctgctctggtgctgcagtatctgagggtgcccctggtggacagagctacctgcctgctgagcaccaagttcaccatctacaacaatatgttctgtgctggatttcatgagggagggagggactcctgtcagggagattctggaggccctcatgtgacagaggtggaaggcaccagcttcctgactggcatcatctcttggggggaggaatgtgctatgaaggggaaatatggaatctataccaaggtgtccagatatgtcaactggatcaaggagaaaaccaagctgacctga

SEQ ID NO: 11 - DNA, 4404 bp, Artificial Sequence
  recombinant fVIII
atgcagctggaactgtctacctgtgtgtttctgtgtctgctgcctctggggttttctgctatcaggagatactatctgggagctgtggagctgtcctgggactacaggcagtctgagctgctgagagaactgcatgtggataccagattcccagctacagctccaggagctctgcctctgggcccatctgtgctgtacaagaaaacagtctttgtggagtttacagaccagctgttctctgtggccaggccaagaccaccttggatgggactgctgggaccaaccatccaggctgaggtgtatgatacagtggtggtgaccctgaaaaacatggcctcccatcctgtgagcctgcatgctgtgggggtgtccttctggaagtcctctgagggagctgagtatgaagaccatacctcccagagggagaaagaagatgataaggtgctgcctggcaaaagccagacctatgtctggcaggtgctgaaggagaatggaccaactgcttctgacccaccatgcctgacctactcttatctgtcccatgtggatctggtgaaggacctgaattctggactgattggagctctgctggtgtgtagagagggaagcctgaccagagaaagaacccagaacctgcatgagtttgtcctgctgtttgctgtgtttgatgaagggaagagctggcactctgccaggaatgactcctggaccagagctatggatccagctcctgctagagctcagcctgctatgcacacagtcaatggctatgtgaataggtctctgccaggactgattggctgccataagaaatctgtctattggcatgtgattggaatgggcaccagccctgaggtgcattctatcttcctggaaggccacacctttctggtcaggcaccatagacaggcctctctggagatctcccctctgaccttcctgacagctcagacctttctgatggacctggggcagttcctgctgttttgccatatctcttcccaccatcatggaggaatggaggctcatgtcagggtggaatcctgtgctgaggaaccacagctgagaagaaaggctgatgaggaagaggactatgatgataacctgtatgactctgatatggatgtggtgaggctggatggggatgatgtcagccctttcatccagatcaggtctgtggccaagaaacatccaaagacctgggtccactacattgctgctgaagaggaagattgggactatgcccccctggtgctggctcctgatgatagatcctacaaaagccagtatctgaacaatgggccccagaggattggaaggaagtacaagaaagtgaggttcatggcctatacagatgagacctttaagaccagagaggctatccagcatgaatctgggatcctgggacctctgctgtatggagaagtgggggataccctgctgatcatcttcaagaaccaggcctccaggccatacaatatctatccccatggcatcacagatgtgagaccactgtacagcaggagactgcccaagggggtcaaacacctgaaggatttccccatcctgcctggagagatctttaagtataaatggacagtcacagtggaagatgggcctaccaagtctgatccaaggtgcctgaccagatactatagctcttttgtgaacatggagagagacctggcttctggactgattggacccctgctgatctgttacaaagagtctgtggaccagaggggcaaccagatcatgtctgataagagaaatgtcatcctgttctctgtgtttgatgagaacaggagctggtacctgacagagaacatccagaggttcctgccaaatccagctggagtgcagctggaggacccagaatttcaggcttccaacatcatgcatagcatcaatggctatgtgtttgatagcctgcagctgtctgtctgcctgcatgaggtggcctactggtatatcctgtccattggagctcagacagacttcctgtctgtgttctttagtgggtacacctttaagcataaaatggtgtatgaggataccctgaccctgttccccttttctggggagacagtgttcatgtccatggaaaaccctggcctgtggatcctggggtgccacaactctgacttcaggaatagaggaatgacagccctgctgaaagtgtccagctgtgataagaatacaggggattactatgaggactcttatgaagatatctctgcttatctgctgagcaagaacaatgccattgagcccaggtcttttgctcagaactccagacctccatctgcttctgctcctaagccacctgtgctgagaagacatcagagggacatctccctgcctaccttccagccagaggaagataaaatggactatgatgatatcttcagcacagagaccaagggggaagattttgacatctatggagaggatgaaaaccaggatccaagatccttccagaagagaaccagacactactttattgctgctgtggagcagctgtgggactatgggatgtctgaaagcccaagggccctgaggaacagagctcagaatggagaggtgcccagattcaagaaagtggtgttcagagagtttgctgatggcagctttacccagccatcttacaggggggagctgaacaagcatctggggctgctgggaccctatatcagagctgaggtggaagataacatcatggtgaccttcaagaatcaggcttctaggccctactccttttattcttccctgatctcctaccctgatgatcaggagcagggagctgaacctaggcacaactttgtgcagccaaatgagaccagaacctacttttggaaggtgcagcatcacatggctcccacagaggatgaatttgactgcaaagcttgggcctatttttctgatgtggacctggagaaggatgtgcattctggcctgattgggcctctgctgatctgtagggccaacaccctgaatgctgctcatggaagacaggtcacagtgcaggagtttgctctgttctttaccatctttgatgaaaccaagagctggtacttcacagagaatgtggaaaggaattgcagagccccctgtcatctgcagatggaggaccctaccctgaaggaaaactacaggttccatgccatcaatggatatgtcatggataccctgcctggcctggtcatggctcagaaccagaggatcagatggtacctgctgtctatgggatccaatgagaatatccatagcatccacttctctggccatgtcttttctgtgaggaagaaagaggaatacaaaatggctgtgtacaatctgtatcctggggtctttgagacagtggaaatgctgccaagcaaagtgggaatctggagaattgagtgcctgattggggaacacctgcaggctgggatgagcaccaccttcctggtgtactctaagaaatgtcagaccccactggggatggcctctggacatatcagggacttccagatcacagcttctggacagtatggacagtgggctccaaagctggctagactgcactattctggctccatcaatgcctggtctaccaaagagccattctcctggatcaaggtggacctgctggcccccatgatcatccatggaatcaaaacccagggagctaggcagaagttcagctctctgtacatctcccagtttatcatcatgtatagcctggatgggaagaaatggcagacctacagaggcaattccactgggaccctgatggtcttctttggaaatgtggattcctctggcatcaagcacaacatcttcaatccacccatcattgccaggtacatcaggctgcatcctacccactatagcatcaggtctaccctgagaatggagctgatgggatgtgacctgaacagctgttctatgccactgggcatggagtccaaggctatctctgatgcccagatcacagcttcttcctacttcaccaatatgtttgctacctggtccccaagcaaggctagactgcacctgcagggaagatccaatgcttggagaccccaggtgaacaatcctaaggagtggctgcaggtggacttccagaaaaccatgaaggtcacaggggtgaccacccagggagtgaaatctctgctgacctccatgtatgtcaaggagttcctgatcagctcttcccaggatggccaccagtggaccctgttctttcagaatggcaaggtcaaagtgttccaggggaatcaggactcttttaccccagtggtgaactccctggatcctccactgctgaccaggtacctgagaatccatcctcagagctgggtgcaccagattgctctgagaatggaggtcctgggatgtgaagctcaggacctgtattga

SEQ ID NO: 12 - DNA, 4404 bp, Artificial Sequence
  recombinant fVIII
atgcagctggaactgtctacctgtgtgtttctgtgtctgctgcctctggggttttctgctatccgccgctactatctgggagccgtggagctgtcctgggactacaggcagagcgagctgctgagagaactgcacgtggataccagattcccagctaccgctccaggagctctgcctctgggcccatccgtgctgtacaagaaaaccgtcttcgtggagtttaccgaccagctgttcagcgtggccaggccaagaccaccttggatgggactgctgggaccaaccatccaggctgaggtgtacgataccgtggtcgtgaccctgaaaaacatggcctcccatcccgtgagcctgcacgctgtcggggtgtccttctggaagtccagcgagggagccgagtacgaagaccatacctcccagcgcgagaaagaagacgataaggtgctgcctggcaaaagccagacctatgtctggcaggtgctgaaggagaacggaccaaccgctagcgacccaccatgcctgacctactcttatctgtcccacgtcgatctggtgaaggacctgaattccggactgatcggagctctgctggtgtgtagagagggaagcctgaccagagaaagaacccagaacctgcatgagttcgtcctgctgttcgccgtgtttgacgaagggaagagctggcactctgcccgcaatgactcctggaccagagctatggatccagctcctgctagagctcagcctgctatgcacaccgtcaacggctacgtgaatcggtctctgccaggactgatcggctgccataagaaaagcgtctattggcacgtgatcggaatgggcaccagccccgaggtgcattctatcttcctggaaggccacacctttctggtcaggcaccatagacaggcctctctggagatctcccctctgaccttcctgaccgctcagacctttctgatggacctggggcagttcctgctgttttgccatatctcttcccaccatcacggaggaatggaggctcacgtcagggtggaatcctgtgctgaggaaccacagctgagaagaaaggctgatgaggaagaggactacgacgataacctgtatgacagcgatatggacgtcgtgcgcctggacggcgacgatgtcagccctttcatccagatccggtctgtggccaagaaacatccaaagacctgggtccactacatcgccgctgaagaggaagattgggactatgcccccctggtgctggctcctgacgatagatcctacaaaagccagtatctgaacaatgggccccagcgcatcggacggaagtacaagaaagtgaggttcatggcctataccgacgagacctttaagaccagagaggctatccagcacgaatccgggatcctgggacctctgctgtacggcgaagtgggggataccctgctgatcatcttcaagaaccaggcctccaggccatacaatatctatccccatggcatcaccgacgtgagaccactgtacagcaggagactgcccaagggggtcaaacacctgaaggatttccccatcctgcctggagagatctttaagtataaatggaccgtcaccgtggaagacgggcctaccaagtccgatccacgctgcctgacccggtactatagctctttcgtgaacatggagagagacctggctagcggactgatcggacccctgctgatctgttacaaagagagcgtggaccagaggggcaaccagatcatgtctgataagagaaatgtcatcctgttctccgtgtttgacgagaaccgcagctggtacctgaccgagaacatccagcggttcctgccaaatccagctggagtgcagctggaggacccagaatttcaggcttccaacatcatgcatagcatcaatggctacgtgttcgatagcctgcagctgtctgtctgcctgcacgaggtggcctactggtatatcctgtccatcggcgctcagaccgacttcctgtccgtgttctttagcgggtacacctttaagcataaaatggtgtatgaggataccctgaccctgttccccttttctggcgagaccgtgttcatgtccatggaaaaccctggcctgtggatcctggggtgccacaacagcgacttcaggaatagaggaatgaccgccctgctgaaagtgtccagctgtgataagaataccggcgattactatgaggactcttacgaagatatctccgcttatctgctgagcaagaacaatgccatcgagcccaggtctttcgctcagaactccagacctccaagcgcttctgctcctaagccacctgtgctgagaagacatcagagggacatctccctgcctaccttccagccagaggaagataaaatggactacgacgatatcttcagcaccgagaccaagggggaagattttgacatctatggagaggacgaaaaccaggatccaagatccttccagaagagaaccagacactactttatcgccgctgtggagcagctgtgggactatgggatgtccgaaagcccacgggccctgaggaacagagctcagaatggagaggtgccccgcttcaagaaagtcgtgttccgggagtttgccgacggcagctttacccagccatcttacaggggggagctgaacaagcatctggggctgctgggaccctatatcagagccgaggtcgaagataacatcatggtgaccttcaagaatcaggcttctcgcccctactccttttattcttccctgatctcctaccctgacgatcaggagcagggcgccgaacctaggcacaacttcgtgcagccaaatgagaccagaacctacttttggaaggtgcagcatcacatggctcccaccgaggatgaattcgactgcaaagcttgggcctatttttccgatgtcgacctggagaaggacgtgcatagcggcctgatcgggcctctgctgatctgtcgcgccaacaccctgaatgctgctcacggaagacaggtcaccgtgcaggagttcgctctgttctttaccatctttgacgaaaccaagagctggtacttcaccgagaacgtggaaaggaattgcagagccccctgtcatctgcagatggaggaccctaccctgaaggaaaactacaggttccacgccatcaatggatatgtcatggataccctgcccggcctggtcatggctcagaaccagcgcatccggtggtacctgctgtctatgggatccaacgagaatatccatagcatccacttctctggccatgtcttttccgtgaggaagaaagaggaatacaaaatggccgtgtacaatctgtatcctggggtcttcgagaccgtggaaatgctgccaagcaaagtgggaatctggagaatcgagtgcctgatcggcgaacacctgcaggccgggatgagcaccaccttcctggtgtactctaagaaatgtcagaccccactggggatggcctccggacatatccgcgacttccagatcaccgctagcggacagtacggacagtgggctccaaagctggctagactgcactattctggctccatcaacgcctggtctaccaaagagccattctcctggatcaaggtggacctgctggcccccatgatcatccacggaatcaaaacccagggcgctaggcagaagttcagctctctgtacatctcccagtttatcatcatgtatagcctggacgggaagaaatggcagacctacagaggcaattccaccgggaccctgatggtcttctttggaaacgtggattccagcggcatcaagcacaacatcttcaatccacccatcatcgcccgctacatccggctgcatcctacccactatagcatcaggtctaccctgagaatggagctgatgggatgcgacctgaacagctgttctatgccactgggcatggagtccaaggctatcagcgatgcccagatcaccgcttcttcctacttcaccaatatgtttgctacctggtccccaagcaaggctagactgcacctgcagggaagatccaacgcttggagaccccaggtgaacaatcctaaggagtggctgcaggtcgacttccagaaaaccatgaaggtcaccggggtgaccacccagggagtgaaatctctgctgacctccatgtacgtcaaggagttcctgatcagctcttcccaggacggccaccagtggaccctgttctttcagaacggcaaggtcaaagtgttccaggggaatcaggactcttttacccccgtcgtgaactccctggatcctccactgctgaccaggtacctgagaatccatcctcagagctgggtgcaccagatcgctctgagaatggaggtcctgggatgcgaagctcaggacctgtattga

SEQ ID NO: 13 - protein, 391 aa, Artificial Sequence
  recombinant promoter sequence
MQIELSTCFFLCLLRFCFSATRRYYLGAVELSWDYMQSDLGELPVDARFPPRVPKSFPFNTSVVYKKTLFVEFTVHLFNIAKPRPPWMGLLGPTIQAEVYDTVVITLKNMASHPVSLHAVGVSYWKASEGAEYDDQTSQREKEDDKVFPGGSHTYVWQVLKENGPMASDPLCLTYSYLSHVDLVKDLNSGLIGALLVCREGSLAKEKTQTLHKFILLFAVFDEGKSWHSETKNSLMQDRDAASARAWPKMHTVNGYVNRSLPGLIGCHRKSVYWHVIGMGTTPEVHSIFLEGHTFLVRNHRQASLEISPITFLTAQTLLMDLGQFLLFCHISSHQHDGMEAYVKVDSCPEEPQLRMKNNEEAEDYDDDLTDSEMDVVRFDDDNSPSFIQIR

SEQ ID NO: 14 - protein, 391 aa, Artificial Sequence
  recombinant promoter sequence
MQLELSTCVFLCLLPLGFSAIRRYYLGAVELSWDYRQSELLRELHVDTRFPATAPGALPLGPSVLYKKTVFVEFTDQLFSVARPRPPWMGLLGPTIQAEVYDTVVVTLKNMASHPVSLHAVGVSFWKSSEGAEYEDHTSQREKEDDKVLPGKSQTYVWQVLKENGPTASDPPCLTYSYLSHVDLVKDLNSGLIGALLVCREGSLTRERTQNLHEFVLLFAVFDEGKSWHSARNDSWTRAMDPAPARAQPAMHTVNGYVNRSLPGLIGCHKKSVYWHVIGMGTSPEVHSIFLEGHTFLVRHHRQASLEISPLTFLTAQTFLMDLGQFLLFCHISSHHHGGMEAHVRVESCAEEPQLRRKADEEEDYDDNLYDSDMDVVRLDGDDVSPFIQIR

SEQ ID NO: 15 - protein, 371 aa, Artificial Sequence
  recombinant promoter sequence
EITRTTLQSDQEEIDYDDTISVEMKKEDFDIYDEDENQSPRSFQKKTRHYFIAAVERLWDYGMSSSPHVLRNRAQSGSVPQFKKVVFQEFTDGSFTQPLYRGELNEHLGLLGPYIRAEVEDNIMVTFRNQASRPYSFYSSLISYEEDQRQGAEPRKNFVKPNETKTYFWKVQHHMAPTKDEFDCKAWAYFSDVDLEKDVHSGLIGPLLVCHTNTLNPAHGRQVTVQEFALFFTIFDETKSWYFTENMERNCRAPCNIQMEDPTFKENYRFHAINGYIMDTLPGLVMAQDQRIRWYLLSMGSNENIHSIHFSGHVFTVRKKEEYKMALYNLYPGVFETVEMLPSKAGIWRVECLIGEHLHAGMSTLFLVYSN

SEQ ID NO: 16 - protein, 371 aa, Artificial Sequence
  recombinant promoter sequence
DISLPTFQPEEDKMDYDDIFSTETKGEDFDIYGEDENQDPRSFQKRTRHYFIAAVEQLWDYGMSESPRALRNRAQNGEVPRFKKVVFREFADGSFTQPSYRGELNKHLGLLGPYIRAEVEDNIMVTFKNQASRPYSFYSSLISYPDDQEQGAEPRHNFVQPNETRTYFWKVQHHMAPTEDEFDCKAWAYFSDVDLEKDVHSGLIGPLLICRANTLNAAHGRQVTVQEFALFFTIFDETKSWYFTENVERNCRAPCHLQMEDPTLKENYRFHAINGYVMDTLPGLVMAQNQRIRWYLLSMGSNENIHSIHFSGHVFSVRKKEEYKMAVYNLYPGVFETVEMLPSKVGIWRIECLIGEHLQAGMSTTFLVYSK

SEQ ID NO: 17 - protein, 461 aa, Artificial Sequence [sequence omitted]

SEQ ID NO: 18 - protein, 461 aa, Artificial Sequence
  recombinant fIX
MQRVNMIMAESPGLITICLLGYLLSAECTVFLDHENANKILNRPKRYNSGKLEEFVQGNLERECMEEKCSFEEAREVFENTERTTEFWKQYVDGDQCESNPCLNGGSCKDDINSYECWCPFGFEGKNCELDVTCNIKNGRCEQFCKNSADNKVVCSCTEGYRLAENQKSCEPAVPFPCGRVSVSQTSKLTRAEAVFPDVDYVNSTEAETILDNITQSTQSFNDFTRVVGGEDAKPGQFPWQVVLNGKVDAFCGGSIVNEKWIVTAAHCVETGVKITVVAGEHNIEETEHTEQKRNVIRIIPHHNYNAAINKYNHDIALLELDEPLVLNSYVTPICIADKEYTNIFLKFGSGYVSGWGRVFHKGRSALVLQYLRVPLVDRATCLLSTKFTIYNNMFCAGFHEGGRDSCQGDSGGPHVTEVEGTSFLTGIISWGEECAMKGKYGIYTKVSRYVNWIKEKTKLT

SEQ ID NO: 19 - protein, 461 aa, Artificial Sequence
  recombinant fIX
MQRVNMIMAESPGLITICLLGYLLSAECTVFLDHENANKILNRPKRYNSGKLEEFVQGNLERECMEEKCSFEEAREVFENTERTTEFWKQYVDGDQCESNPCLNGGSCKDDINSYECWCPFGFEGKNCELDVTCNIKNGRCEQFCKNSADNKVVCSCTEGYRLAENQKSCEPAVPFPCGRVSVSQTSKLTRAETVFPDVDYVNSTEAETILDNITQSTQSFNDFTRVVGGEDAKPGQFPWQVVLNGKVDAFCGGSIVNEKWIVTAAHCVETGVKITVVAGEHNIEETEHTEQKRNVIRIIPHHNYNAAINKYNHDIALLELDEPLVLNSYVTPICIADKEYTNIFLKFGSGYVSGWGRVFHKGRSALVLQYLRVPLVDRATCLLSTKFTIYNNMFCAGFHEGGRDSCQGDSGGPHVTEVEGTSFLTGIISWGEECAMKGKYGIYTKVSRYVNWIKEKTKLT

SEQ ID NO: 20 - DNA, 39 bp, Artificial Sequence
  recombinant promoter sequence
tataaaaggccagcagcagcctgaccacatctcatcctc

SEQ ID NO: 21 - DNA, 38 bp, Artificial Sequence
  recombinant promoter sequence
gttaatttttgtggcccttgcgatgtttgctctggtta

SEQ ID NO: 22 - protein, 14 aa, Artificial Sequence
  recombinant peptide linker
SFSQNPPVLKRHQR

SEQ ID NO: 23 - protein, 24 aa, Artificial Sequence
  recombinant peptide linker
SFAQNSRPPSASAPKPPVLRRHQR

SEQ ID NO: 24 - protein, 4 aa, Artificial Sequence
  recombinant promoter sequence
RHQR

SEQ ID NO: 25 - DNA, 6 bp, Artificial Sequence
  recombinant promoter sequence
gttaat

SEQ ID NO: 26 - DNA, 5 bp, Artificial Sequence
  recombinant promoter sequence
tataa

SEQ ID NO: 27 - DNA, 5 bp, Artificial Sequence
  recombinant promoter sequence
gttaa

SEQ ID NO: 28 - DNA, 4 bp, Artificial Sequence
  recombinant promoter sequence
gtta

SEQ ID NO: 29 - DNA, 3 bp, Artificial Sequence
  recombinant promoter sequence
gtt

SEQ ID NO: 30 - DNA, 5 bp, Artificial Sequence
  recombinant promoter sequence
ttaat

SEQ ID NO: 31 - DNA, 4 bp, Artificial Sequence
  recombinant promoter sequence
ttaa

SEQ ID NO: 32 - DNA, 3 bp, Artificial Sequence
  recombinant promoter sequence
tta

SEQ ID NO: 33 - DNA, 3 bp, Artificial Sequence
  recombinant promoter sequence
aat

SEQ ID NO: 34 - DNA, 56 bp, Artificial Sequence
  recombinant promoter sequence
gttaatttttgtggcccttgcgatgtttgctctggttaataatctcaggacaaaca

SEQ ID NO: 35 - DNA, 55 bp, Artificial Sequence
  recombinant promoter sequence
ttaatttttgtggcccttgcgatgtttgctctggttaataatctcaggacaaaca

SEQ ID NO: 36 - DNA, 54 bp, Artificial Sequence
  recombinant promoter sequence
taatttttgtggcccttgcgatgtttgctctggttaataatctcaggacaaaca

SEQ ID NO: 37 - DNA, 53 bp, Artificial Sequence
  recombinant promoter sequence
aatttttgtggcccttgcgatgtttgctctggttaataatctcaggacaaaca

SEQ ID NO: 38 - DNA, 52 bp, Artificial Sequence
  recombinant promoter sequence
atttttgtggcccttgcgatgtttgctctggttaataatctcaggacaaaca

SEQ ID NO: 39 - DNA, 51 bp, Artificial Sequence
  recombinant promoter sequence
tttttgtggcccttgcgatgtttgctctggttaataatctcaggacaaaca

SEQ ID NO: 40 - DNA, 50 bp, Artificial Sequence
  recombinant promoter sequence
ttttgtggcccttgcgatgtttgctctggttaataatctcaggacaaaca

SEQ ID NO: 41 - DNA, 49 bp, Artificial Sequence
  recombinant promoter sequence
tttgtggcccttgcgatgtttgctctggttaataatctcaggacaaaca

SEQ ID NO: 42 - DNA, 48 bp, Artificial Sequence
  recombinant promoter sequence
ttgtggcccttgcgatgtttgctctggttaataatctcaggacaaaca

SEQ ID NO: 43 - DNA, 18 bp, Artificial Sequence
  recombinant promoter sequence
ataatctcaggacaaaca

SEQ ID NO: 44 - DNA, 47 bp, Artificial Sequence
  recombinant promoter sequence
tgtggcccttgcgatgtttgctctggttaataatctcaggacaaaca

SEQ ID NO: 45 - DNA, 46 bp, Artificial Sequence
  recombinant promoter sequence
gtggcccttgcgatgtttgctctggttaataatctcaggacaaaca

SEQ ID NO: 46 - DNA, 45 bp, Artificial Sequence
  recombinant promoter sequence
tggcccttgcgatgtttgctctggttaataatctcaggacaaaca

SEQ ID NO: 47 - DNA, 43 bp, Artificial Sequence
  recombinant promoter sequence
gcccttgcgatgtttgctctggttaataatctcaggacaaaca

SEQ ID NO: 48 - DNA, 42 bp, Artificial Sequence
  recombinant promoter sequence
cccttgcgatgtttgctctggttaataatctcaggacaaaca

SEQ ID NO: 49 - DNA, 41 bp, Artificial Sequence
  recombinant promoter sequence
ccttgcgatgtttgctctggttaataatctcaggacaaaca

SEQ ID NO: 50 - DNA, 40 bp, Artificial Sequence
  recombinant promoter sequence
cttgcgatgtttgctctggttaataatctcaggacaaaca

SEQ ID NO: 51 - DNA, 55 bp, Artificial Sequence
  recombinant promoter sequence
gttaatttttgtggcccttgcgatgtttgctctggttaataatctcaggacaaac

SEQ ID NO: 52 - DNA, 54 bp, Artificial Sequence
  recombinant promoter sequence
gttaatttttgtggcccttgcgatgtttgctctggttaataatctcaggacaaa

SEQ ID NO: 53 - DNA, 53 bp, Artificial Sequence
  recombinant promoter sequence
gttaatttttgtggcccttgcgatgtttgctctggttaataatctcaggacaa

SEQ ID NO: 54 - DNA, 53 bp, Artificial Sequence; identical to SEQ ID NO: 53
  recombinant promoter sequence

SEQ ID NO: 55 - DNA, 52 bp, Artificial Sequence
  recombinant promoter sequence
gttaatttttgtggcccttgcgatgtttgctctggttaataatctcaggaca

SEQ ID NO: 56 - DNA, 51 bp, Artificial Sequence
  recombinant promoter sequence
gttaatttttgtggcccttgcgatgtttgctctggttaataatctcaggac

SEQ ID NO: 57 - DNA, 50 bp, Artificial Sequence
  recombinant promoter sequence
gttaatttttgtggcccttgcgatgtttgctctggttaataatctcagga

SEQ ID NO: 58 - DNA, 49 bp, Artificial Sequence
  recombinant promoter sequence
gttaatttttgtggcccttgcgatgtttgctctggttaataatctcagg

SEQ ID NO: 59 - DNA, 48 bp, Artificial Sequence
  recombinant promoter sequence
gttaatttttgtggcccttgcgatgtttgctctggttaataatctcag

SEQ ID NO: 60 - DNA, 47 bp, Artificial Sequence
  recombinant promoter sequence
gttaatttttgtggcccttgcgatgtttgctctggttaataatctca

SEQ ID NO: 61 - DNA, 46 bp, Artificial Sequence
  recombinant promoter sequence
gttaatttttgtggcccttgcgatgtttgctctggttaataatctc

SEQ ID NO: 62 - DNA, 45 bp, Artificial Sequence
  recombinant promoter sequence
gttaatttttgtggcccttgcgatgtttgctctggttaataatct

SEQ ID NO: 63 - DNA, 44 bp, Artificial Sequence
  recombinant promoter sequence
gttaatttttgtggcccttgcgatgtttgctctggttaataatc

SEQ ID NO: 64 - DNA, 43 bp, Artificial Sequence
  recombinant promoter sequence
gttaatttttgtggcccttgcgatgtttgctctggttaataat

SEQ ID NO: 65 - DNA, 42 bp, Artificial Sequence
  recombinant promoter sequence
gttaatttttgtggcccttgcgatgtttgctctggttaataa

SEQ ID NO: 66 - DNA, 55 bp, Artificial Sequence; identical to SEQ ID NO: 51
  recombinant promoter sequence

SEQ ID NO: 67 - DNA, 53 bp, Artificial Sequence
  recombinant promoter sequence
ttaatttttgtggcccttgcgatgtttgctctggttaataatctcaggacaaa

SEQ ID NO: 68 - DNA, 51 bp, Artificial Sequence
  recombinant promoter sequence
taatttttgtggcccttgcgatgtttgctctggttaataatctcaggacaa

SEQ ID NO: 69 - DNA, 49 bp, Artificial Sequence
  recombinant promoter sequence
aatttttgtggcccttgcgatgtttgctctggttaataatctcaggaca

SEQ ID NO: 70 - DNA, 47 bp, Artificial Sequence
  recombinant promoter sequence
atttttgtggcccttgcgatgtttgctctggttaataatctcaggac

SEQ ID NO: 71 - DNA, 45 bp, Artificial Sequence
  recombinant promoter sequence
tttttgtggcccttgcgatgtttgctctggttaataatctcagga

SEQ ID NO: 72 - DNA, 43 bp, Artificial Sequence
  recombinant promoter sequence
ttttgtggcccttgcgatgtttgctctggttaataatctcagg

SEQ ID NO: 73 - DNA, 41 bp, Artificial Sequence
  recombinant promoter sequence
tttgtggcccttgcgatgtttgctctggttaataatctcag

SEQ ID NO: 74 - DNA, 39 bp, Artificial Sequence
  recombinant promoter sequence
ttgtggcccttgcgatgtttgctctggttaataatctca

SEQ ID NO: 75 - DNA, 37 bp, Artificial Sequence
  recombinant promoter sequence
tgtggcccttgcgatgtttgctctggttaataatctc

SEQ ID NO: 76 - DNA, 35 bp, Artificial Sequence
  recombinant promoter sequence
gtggcccttgcgatgtttgctctggttaataatct

SEQ ID NO: 77 - DNA, 33 bp, Artificial Sequence
  recombinant promoter sequence
tggcccttgcgatgtttgctctggttaataatc

SEQ ID NO: 78 - DNA, 30 bp, Artificial Sequence
  recombinant promoter sequence
gcccttgcgatgtttgctctggttaataat

SEQ ID NO: 79 - DNA, 28 bp, Artificial Sequence
  recombinant promoter sequence
cccttgcgatgtttgctctggttaataa

SEQ ID NO: 80 - DNA, 26 bp, Artificial Sequence
  recombinant promoter sequence
ccttgcgatgtttgctctggttaata

SEQ ID NO: 81 - DNA, 24 bp, Artificial Sequence
  recombinant promoter sequence
cttgcgatgtttgctctggttaat

SEQ ID NO: 82 - DNA, 54 bp, Artificial Sequence
  recombinant promoter sequence
ttaatttttgtggcccttgcgatgtttgctctggttaataatctcaggacaaac

SEQ ID NO: 83 - DNA, 52 bp, Artificial Sequence
  recombinant promoter sequence
taatttttgtggcccttgcgatgtttgctctggttaataatctcaggacaaa

SEQ ID NO: 84 - DNA, 50 bp, Artificial Sequence
  recombinant promoter sequence
aatttttgtggcccttgcgatgtttgctctggttaataatctcaggacaa

SEQ ID NO: 85 - DNA, 49 bp, Artificial Sequence
  recombinant promoter sequence
atttttgtggcccttgcgatgtttgctctggttaataatctcaggacaa

SEQ ID NO: 86 - DNA, 47 bp, Artificial Sequence
  recombinant promoter sequence
tttttgtggcccttgcgatgtttgctctggttaataatctcaggaca

SEQ ID NO: 87 - DNA, 45 bp, Artificial Sequence
  recombinant promoter sequence
ttttgtggcccttgcgatgtttgctctggttaataatctcaggac

SEQ ID NO: 88 - DNA, 43 bp, Artificial Sequence
  recombinant promoter sequence
tttgtggcccttgcgatgtttgctctggttaataatctcagga

SEQ ID NO: 89 - DNA, 41 bp, Artificial Sequence
  recombinant promoter sequence
ttgtggcccttgcgatgtttgctctggttaataatctcagg

SEQ ID NO: 90 - DNA, 39 bp, Artificial Sequence
  recombinant promoter sequence
tgtggcccttgcgatgtttgctctggttaataatctcag

SEQ ID NO: 91 - DNA, 36 bp, Artificial Sequence
  recombinant promoter sequence
tggcccttgcgatgtttgctctggttaataatctca

SEQ ID NO: 92 - DNA, 34 bp, Artificial Sequence
  recombinant promoter sequence
ggcccttgcgatgtttgctctggttaataatctc

SEQ ID NO: 93 - DNA, 32 bp, Artificial Sequence
  recombinant promoter sequence
gcccttgcgatgtttgctctggttaataatct

SEQ ID NO: 94 - DNA, 30 bp, Artificial Sequence
  recombinant promoter sequence
cccttgcgatgtttgctctggttaataatc

SEQ ID NO: 95 - DNA, 28 bp, Artificial Sequence
  recombinant promoter sequence
ccttgcgatgtttgctctggttaataat

SEQ ID NO: 96 - DNA, 26 bp, Artificial Sequence
  recombinant promoter sequence
cttgcgatgtttgctctggttaataa

SEQ ID NO: 97 - DNA, 17 bp, Artificial Sequence
  recombinant promoter sequence
cggaggagcaaacaggg

SEQ ID NO: 98 - DNA, 28 bp, Artificial Sequence
  recombinant promoter sequence
cggaggagcaaacaggggctaagtccac

SEQ ID NO: 99 - DNA, 27 bp, Artificial Sequence
  recombinant promoter sequence
ggctgctggtgaatattaaccaaggtc

SEQ ID NO: 100 - DNA, 71 bp, Artificial Sequence
  recombinant promoter sequence
ggggaggctgctggtgaatattaaccaaggtcaccccagttatcggaggagcaaacaggggctaagtccac

SEQ ID NO: 101 - DNA, 71 bp, Artificial Sequence
  recombinant promoter sequence
ggggaggctgctggtgaatattaaccaaggtcaccccagttatcggaggagcaaacagggactaagtccac

SEQ ID NO: 102 - DNA, 220 bp, Artificial Sequence
  recombinant promoter sequence
ggggaggctgctggtgaatattaaccaaggtcaccccagttatcggaggagcaaacaggggctaagtccactaggttaatcattaagtcgttaatttttgtggcccttgcgatgtttgctctggttaataatctcaggacaaacagaggttaataattttccagatctctctgagcaatagtataaaaggccagcagcagcctgaccacatctcatcctc

SEQ ID NO: 103 - DNA, 171 bp, Artificial Sequence
  recombinant promoter sequence
cggaggagcaaacaggggctaagtcgttaatcattaagtcgttaatttttgtggcccttgcgatgtttgctctggttaataatctcaggacaaacagaggttaataattttccagatctctctgagcaatagtataaaaggccagcagcagcctgaccacatctcatcctc

SEQ ID NO: 104 - DNA, 173 bp, Artificial Sequence
  recombinant promoter sequence
ggctgctggtgaatattaaccaaggtcgttaatcattaagtcgttaatttttgtggcccttgcgatgtttgctctggttaataatctcaggacaaacagaggttaataattttccagatctctctgagcaatagtataaaaggccagcagcagcctgaccacatctcatcctc

SEQ ID NO: 105 - DNA, 146 bp, Artificial Sequence
  recombinant promoter sequence
ggggaggctgctggtgaatattaaccaaggtcaccccagttatcggaggagcaaacaggggctaagtccacgaggttaataattttccagatctctctgagcaatagtataaaaggccagcagcagcctgaccacatctcatcctc

SEQ ID NO: 106 - DNA, 129 bp, Artificial Sequence
  recombinant promoter sequence
ggctgctggtgaatattaaccaaggtcatcggaggagcaaacagggactaagtcgaggttaataattttccagatctctctgagcaatagtataaaaggccagcagcagcctgaccacatctcatcctc

SEQ ID NO: 107 - DNA, 142 bp, Artificial Sequence
  recombinant promoter sequence
ggctgctggtgaatattaaccaaggtccccttgctggttaataatctcagttaatttgtttgcacaaacacggaggagcaaacaggggaggttaataattttctataaaaggccagcagcagcctgaccacatctcatcctc

SEQ ID NO: 108 - DNA, 146 bp, Artificial Sequence
  recombinant promoter sequence
ggggaggctgctggtgaatattaaccaaggtcaccccagttatcggaggagcaaacagggactaagtccacgaggttaataattttccagatctctctgagcaatagtataaaaggccagcagcagcctgaccacatctcatcctc

SEQ ID NO: 109 - DNA, 8 bp, Artificial Sequence
  recombinant promoter sequence
tcatcctc

SEQ ID NO: 110 - DNA, 24 bp, Artificial Sequence
  recombinant promoter sequence
ggccagcagcagcctgaccacatc

SEQ ID NO: 111 - DNA, 71 bp, Artificial Sequence; identical to SEQ ID NO: 100
  recombinant promoter sequence

SEQ ID NO: 112 - DNA, 255 bp, Artificial Sequence
  recombinant promoter sequence
gttaatcattaagtcgttaatcattaacttaggtcaaaggtcagacaatgttgactctcgttaatgattaaccggaattgttgacttgaggttaataattttccagatctctctgagcaatagtataaaaggccagcagcagcctgaccacatctcatcctcctctaaggtaaatataaaatttttaagtgtataatgtgttaaactactgattctaattgtttgtgtattttagattccaacctatggaactga

SEQ ID NO: 113 - DNA, 94 bp, Artificial Sequence
  recombinant promoter sequence
gttaatttttaaaaagcagtcaaaagtccaagtggcccttgcgagcatttactctctctgtttgctctggttaataatctcaggagcacaaaca

SEQ ID NO: 114 - DNA, 43 bp, Artificial Sequence
  recombinant promoter sequence
gaggttaataattttccagatctctctgagcaatagtataaaa

SEQ ID NO: 115 - DNA, 55 bp, Artificial Sequence
  recombinant promoter sequence
agtcatatgtttgctcactgaaggttactagttaacaggcatcccttaaacagga

SEQ ID NO: 116 - DNA, 108 bp, Artificial Sequence
  recombinant promoter sequence
gttaatcattaacttaaaaagcagtcaaaagtccaaaggtcaaaggtcagagcatttactctctccaatgttgactctcgttaatgattaaggagcaattgttgactt

SEQ ID NO: 117 - DNA, 72 bp, Artificial Sequence
  recombinant promoter sequence
gttaatcattaacttaggtcaaaggtcagacaatgttgactctcgttaatgattaaccggaattgttgactt

SEQ ID NO: 118 - DNA, 151 bp, Artificial Sequence
  recombinant promoter sequence
gttaatcattaacttaaaaagcagtcaaaagtccaaaggtcaaaggtcagagcatttactctctccaatgttgactctcgttaatgattaaggagcaattgttgacttgaggttaataattttccagatctctctgagcaatagtataaaa

SEQ ID NO: 119 - DNA, 115 bp, Artificial Sequence
  recombinant promoter sequence
gttaatcattaacttaggtcaaaggtcagacaatgttgactctcgttaatgattaaccggaattgttgacttgaggttaataattttccagatctctctgagcaatagtataaaa

SEQ ID NO: 120 - DNA, 152 bp, Artificial Sequence
  recombinant promoter sequence
gttaatcattaagtcgttaatttttaaaaagcagtcaaaagtccaagtggcccttgcgagcatttactctctctgtttgctctggttaataatctcaggagcacaaacagaggttaataattttccagatctctctgagcaatagtataaaa

SEQ ID NO: 121 - DNA, 150 bp, Artificial Sequence
  recombinant promoter sequence
tgggcggagtgtcgttaatttttaaaaagcagtcaaaagtccaagtggcccttgcgagcatttactctctctgtttgctctggttaataatctcaggagcacaaacagaggttaataattttccagatctctctgagcaatagtataaaa

SEQ ID NO: 122 - DNA, 43 bp, Artificial Sequence
  recombinant promoter sequence
cccttgctggttaataatctcagttaatttgtttgcacaaaca

SEQ ID NO: 123 - protein, 1467 aa, Artificial Sequence
  recombinant fVIII
MQLELSTCVFLCLLPLGFSAIRRYYLGAVELSWDYRQSELLRELHVDTRFPATAPGALPLGPSVLYKKTVFVEFTDQLFSVARPRPPWMGLLGPTIQAEVYDTVVVTLKNMASHPVSLHAVGVSFWKSSEGAEYEDHTSQREKEDDKVLPGKSQTYVWQVLKENGPTASDPPCLTYSYLSHVDLVKDLNSGLIGALLVCREGSLTRERTQNLHEFVLLFAVFDEGKSWHSARNDSWTRAMDPAPARAQPAMHTVNGYVNRSLPGLIGCHKKSVYWHVIGMGTSPEVHSIFLEGHTFLVRHHRQASLEISPLTFLTAQTFLMDLGQFLLFCHISSHHHGGMEAHVRVESCAEEPQLRRKADEEEDYDDNLYDSDMDVVRLDGDDVSPFIQIRSVAKKHPKTWVHYIAAEEEDWDYAPLVLAPDDRSYKSQYLNNGPQRIGRKYKKVRFMAYTDETFKTREAIQHESGILGPLLYGEVGDTLLIIFKNQASRPYNIYPHGITDVRPLYSRRLPKGVKHLKDFPILPGEIFKYKWTVTVEDGPTKSDPRCLTRYYSSFVNMERDLASGLIGPLLICYKESVDQRGNQIMSDKRNVILFSVFDENRSWYLTENIQRFLPNPAGVQLEDPEFQASNIMHSINGYVFDSLQLSVCLHEVAYWYILSIGAQTDFLSVFFSGYTFKHKMVYEDTLTLFPFSGETVFMSMENPGLWILGCHNSDFRNRGMTALLKVSSCDKNTGDYYEDSYEDISAYLLSKNNAIEPRSFAQNSRPPSASAPKPPVLRRHQRDISLPTFQPEEDKMDYDDIFSTETKGEDFDIYGEDENQDPRSFQKRTRHYFIAAVEQLWDYGMSESPRALRNRAQNGEVPRFKKVVFREFADGSFTQPSYRGELNKHLGLLGPYIRAEVEDNIMVTFKNQASRPYSFYSSLISYPDDQEQGAEPRHNFVQPNETRTYFWKVQHHMAPTEDEFDCKAWAYFSDVDLEKDVHSGLIGPLLICRANTLNAAHGRQVTVQEFALFFTIFDETKSWYFTENVERNCRAPCHLQMEDPTLKENYRFHAINGYVMDTLPGLVMAQNQRIRWYLLSMGSNENIHSIHFSGHVFSVRKKEEYKMAVYNLYPGVFETVEMLPSKVGIWRIECLIGEHLQAGMSTTFLVYSKKCQTPLGMASGHIRDFQITASGQYGQWAPKLARLHYSGSINAWSTKEPFSWIKVDLLAPMIIHGIKTQGARQKFSSLYISQFIIMYSLDGKKWQTYRGNSTGTLMVFFGNVDSSGIKHNIFNPPIIARYIRLHPTHYSIRSTLRMELMGCDLNSCSMPLGMESKAISDAQITASSYFTNMFATWSPSKARLHLQGRSNAWRPQVNNPKEWLQVDFQKTMKVTGVTTQGVKSLLTSMYVKEFLISSSQDGHQWTLFFQNGKVKVFQGNQDSFTPVVNSLDPPLLTRYLRIHPQSWVHQIALRMEVLGCEAQDLY

SEQ ID NO: 124 - DNA, 1386 bp, Artificial Sequence
  recombinant promoter sequence
atgcagagggtcaatatgatcatggctgaatctcctgggctgatcaccatttgcctgctgggatacctgctgtctgctgagtgtacagtgttcctggaccatgagaatgccaataagatcctgaacaggcccaaaagatacaattctggaaagctggaggaatttgtgcagggcaacctggagagggaatgcatggaggaaaagtgtagctttgaggaagctagggaggtgtttgaaaacacagagaggaccacagaattctggaagcagtatgtggatggagatcagtgtgagtccaacccctgtctgaatggagggtcttgcaaagatgatatcaactcctatgagtgctggtgtccttttggatttgaaggcaaaaattgtgagctggatgtgacctgtaacatcaagaatggcaggtgtgagcagttctgtaaaaactctgctgataataaggtggtctgcagctgtacagaaggctataggctggctgagaaccagaagagctgtgaaccagctgtgcccttcccttgtgggagggtgtctgtcagccagacctctaagctgaccagagctgagactgtgttcccagatgtggattatgtcaactccacagaggctgaaaccatcctggacaacatcacccagtctacccagtccttcaatgactttaccagagtggtgggaggagaggatgccaaaccaggccagttcccctggcaggtggtcctgaatgggaaggtggatgctttttgtgggggatccattgtgaatgagaaatggattgtcacagctgctcactgtgtggagacaggggtcaagatcactgtggtggctggagagcacaacattgaggaaacagaacatactgagcagaagaggaatgtgatcagaatcatccctcaccataactacaatgctgctatcaacaaatataatcatgacattgccctgctggaactggatgagcctctggtgctgaacagctatgtcaccccaatctgcattgctgacaaagagtataccaatatcttcctgaagtttggatctggatatgtgtctggatggggaagggtcttccacaagggcaggtctgccctggtgctgcagtatctgagggtgcctctggtggacagagctacctgcctgctgtctaccaagttcaccatctacaacaatatgttctgtgctggatttcatgagggaggcagggactcctgtcagggggattctggaggcccacatgtgacagaggtggaaggcaccagcttcctgactggcatcatctcttggggggaggaatgtgctatgaaggggaaatatggaatctacaccaaagtgagcaggtatgtgaactggatcaaagagaagaccaaactgacctga

SEQ ID NO: 125 - DNA, 4404 bp, Artificial Sequence
  recombinant promoter sequence
atgcagctggagctctcaacctgtgtgttcctctgcctgctccccctgggattttcagctatcaggagatactatctgggagcagtggaactgtcctgggactacaggcagtcagagctgctcagagaactgcatgtggatactaggttccctgcaacagctcctggagcactgccactgggaccttcagtgctgtacaagaaaactgtctttgtggagtttacagaccagctgttcagtgtggccaggcccaggcccccctggatggggctgctgggacccaccatccaggctgaagtgtatgatactgtggtggtgaccctgaaaaacatggcctctcatccagtcagcctgcatgctgtgggagtgagcttctggaagagcagtgagggagctgagtatgaagaccatacctcacagagggagaaagaagatgataaggtgctgccaggaaaaagccagacctatgtgtggcaggtgctgaaggagaatggccctacagcttcagatcctccctgcctcacatactcttatctgagccatgtggatctggtgaaggacctcaatagtggcctgattggggcactgctggtgtgcagagaggggtccctcacaagggaaagaactcagaacctgcatgagtttgtcctgctctttgctgtgtttgatgagggaaagtcctggcactcagcaaggaatgacagctggaccagggctatggacccagcaccagccagagctcagccagctatgcacactgtcaatggctatgtgaataggtccctgcctggactcattggctgccataagaaatcagtctattggcatgtgattggaatgggcaccagcccagaggtgcattccatcttcctggaaggccacacatttctggtcaggcaccatagacaggccagcctggagatcagcccactgactttcctcacagcacagacatttctgatggacctggggcagttcctgctcttttgccatatctcaagtcaccatcatggagggatggaggctcatgtcagggtggaaagctgtgcagaggaacctcagctgaggaggaaggcagatgaggaagaggactatgatgataacctgtatgactcagatatggatgtggtgaggctggatggagatgatgtcagcccattcatccagatcaggtcagtggctaagaaacaccctaagacctgggtccactacattgcagctgaagaggaagattgggactatgcacccctggtgctggccccagatgatagaagttacaaatctcagtatctgaacaatgggccccagaggattggaaggaagtacaagaaagtgaggttcatggcttatactgatgagacctttaagacaagagaggcaatccagcatgaaagtggcatcctgggaccactgctctatggagaagtgggggataccctgctcatcatcttcaagaaccaggcctcaaggccttacaatatctatccccatggcatcacagatgtgaggcctctctacagcaggagactgcccaagggagtcaaacacctcaaggatttccccatcctgccaggggaaatcttcaagtataaatggacagtcactgtggaagatgggccaactaagtcagatcctaggtgcctgaccaggtactattctagctttgtgaacatggagagggacctggcttcaggactgattggacctctgctcatctgctacaaagaatcagtggaccagaggggcaaccagatcatgagtgataagagaaatgtcatcctgttctcagtgtttgatgagaataggagttggtatctgacagaaaacatccagaggttcctgcctaatcctgcaggagtgcagctggaggacccagaatttcaggcttcaaacatcatgcatagtatcaatggctatgtgtttgatagtctgcagctctctgtctgcctgcatgaggtggcctactggtatatcctcagcattggagctcagactgacttcctgagtgtgttcttttcaggctacacattcaagcataagatggtctatgaagataccctgacactcttccccttttctggggagactgtgtttatgagcatggaaaacccaggcctgtggattctggggtgccacaacagtgacttcaggaatagagggatgactgctctgctcaaagtgtcctcatgtgataagaatactggagattactatgaggactcttatgaagatatcagtgcatatctgctctccaaaaacaatgccattgagcccaggtcatttgctcagaacagtagaccaccttctgcaagtgcaccaaagcctccagtgctgaggagacaccagagggacatcagcctgccaaccttccagcctgaggaagataaaatggactatgatgatatcttctccactgagaccaagggggaagattttgacatctatggagaggatgaaaaccaggaccccaggtccttccagaagaggaccagacactactttattgcagctgtggagcagctgtgggactatggcatgtctgaatcacctagagctctgaggaacagagcacagaatggggaggtgcccaggttcaagaaagtggtgttcagagaatttgcagatggctcttttacccagcctagctacaggggggagctcaacaagcatctggggctgctgggaccctatatcagagcagaggtggaagataacatcatggtgacattcaagaatcaggcctcaagaccctacagtttttatagttctctgatcagctacccagatgatcaggagcagggggctgaaccaaggcacaactttgtgcagcctaatgagacaagaacttacttttggaaggtccagcatcacatggctcccacagaggatgagtttgactgcaaggcctgggcatatttttctgatgtggacctggagaaggatgtgcatagtggcctcattgggccactgctcatctgcagggcaaacacactgaatgctgcacatggcaggcaggtcactgtgcaggagtttgccctgttctttacaatctttgatgaaactaagtcctggtacttcacagagaatgtggaaaggaattgcagagccccctgccatctccagatggaggacccaactctgaaggaaaactacaggttccatgctatcaatggatatgtcatggatacactgccaggcctggtgatggcacagaaccagaggatcaggtggtatctgctcagcatggggtccaatgagaatatccattctatccacttctcaggacatgtcttttcagtgaggaagaaagaggaatataaaatggctgtgtacaatctgtatccaggggtctttgagacagtggaaatgctgcctagcaaagtggggatctggagaattgagtgcctcattggagaacacctgcaggcagggatgtccaccacatttctggtgtactcaaagaaatgccagactcccctggggatggcaagtggacatatcagggacttccagatcactgcatcaggacagtatggacagtgggcaccaaagctggctaggctccactatagtggctctatcaatgcttggagtaccaaagagcctttctcttggatcaaggtggatctgctggcccccatgatcatccatggaatcaaaacacagggagctagacagaagttcagctccctgtacatcagtcagtttatcatcatgtattctctggatgggaagaaatggcagacctacaggggcaatagcactgggacactgatggtcttctttggaaatgtggattcaagtggcatcaagcacaacatcttcaatcctcccatcattgccaggtacatcagactgcatcccacacactattcaatcaggagtactctcagaatggagctgatggggtgtgacctcaacagctgctccatgccactgggaatggaatccaaggcaatctcagatgcccagatcactgcttctagctacttcaccaatatgtttgcaacatggtcacccagtaaagcaaggctgcacctccagggaaggtccaatgcttggagaccccaggtgaacaatccaaaggagtggctgcaggtggactttcagaaaaccatgaaggtcacaggggtgactacccagggagtgaaaagtctgctcacctctatgtatgtcaaggagttcctgatctcctcaagtcaggatggccaccagtggacactgttctttcagaatggcaaggtcaaagtgttccaggggaatcaggacagctttacaccagtggtgaacagcctggacccccctctgctcactagatatctgagaatccatccacagagctgggtgcaccagattgcactcagaatggaggtcctgggctgtgaagcccaggacctgtattga

SEQ ID NO: 126 - DNA, 4374 bp, Artificial Sequence
  recombinant promoter sequence
atgcagattgagctcagcacctgcttctttctgtgcctgctcaggttctgcttttcagccacaaggagatactatctgggagctgtggaactgtcatgggattacatgcagagtgacctgggagagctccctgtggatgctaggttccccccaagggtcccaaagtctttcccttttaataccagtgtggtctataagaaaacactctttgtggaatttactgatcacctgttcaacattgcaaagccaaggcctccctggatgggactgctgggacctaccatccaggctgaggtgtatgacactgtggtcatcacactgaaaaacatggcatctcaccctgtcagcctgcatgcagtgggagtcagctactggaaggcttcagaaggggcagagtatgatgatcagacaagccagagagaaaaagaggatgataaggtgttcccaggagggagccatacttatgtgtggcaggtcctgaaggagaatggcccaatggccagtgacccactgtgcctcacctactcatatctgagtcatgtggacctggtcaaggatctcaactcaggcctgattggggcactgctggtgtgcagggaaggctcactggccaaggagaaaacccagacactgcataagttcatcctgctctttgctgtgtttgatgaagggaaatcttggcacagtgagaccaagaacagtctgatgcaggacagggatgctgcttctgccagagcttggcccaagatgcacacagtgaatggatatgtcaataggtccctgccaggactcattggctgccacagaaagtcagtgtattggcatgtcattggaatgggcaccacaccagaagtgcacagcatcttcctggaggggcatacctttctggtcaggaaccacaggcaggccagcctggagatcagcccaatcaccttcctgacagcccagactctgctcatggatctggggcagttcctgctcttttgccacatcagctcccaccagcatgatggaatggaggcatatgtgaaagtggactcctgcccagaggaaccacagctgaggatgaagaacaatgaggaagctgaagactatgatgatgacctgacagactcagagatggatgtggtcaggtttgatgatgataacagcccctcctttatccagatcagaagtgtggccaagaaacacccaaagacatgggtccattacattgcagctgaggaagaggactgggattatgcacctctggtgctggccccagatgatagatcctacaaatcacagtatctgaacaatggaccccagaggattggcagaaagtacaagaaagtgaggttcatggcctatactgatgaaacatttaagactagagaagctatccagcatgagtcaggcatcctgggaccactgctctatggagaagtgggggacaccctgctcatcatcttcaagaaccaggcttccaggccatacaatatctatcctcatggcatcacagatgtgagaccactctactcaaggagactgcctaagggagtcaaacacctcaaggacttccctatcctgccaggggaaatctttaagtataaatggactgtgacagtggaggatgggcccactaagagtgacccaaggtgcctgaccagatactattcaagttttgtgaatatggaaagggatctggcatcaggactgattggacctctgctcatctgctacaaagagagtgtggatcagaggggcaaccagatcatgtcagacaagaggaatgtgatcctgttcagtgtctttgatgaaaacaggtcttggtatctgacagagaacatccagagattcctgccaaatcctgcaggggtgcagctggaagatccagagtttcaggcctcaaacatcatgcatagtatcaatggatatgtgtttgacagtctgcagctctctgtgtgcctgcatgaagtggcctactggtatatcctgtccattggagctcagacagatttcctgagtgtgttcttttcaggctacacttttaagcataaaatggtctatgaggacacactgactctcttcccttttagtggggaaacagtgtttatgagcatggagaatccagggctgtggattctgggatgccacaacagtgatttcaggaatagaggcatgactgctctgctcaaagtgtctagctgtgacaagaacacaggggactactatgaagattcttatgaggacatcagtgcttatctgctctccaaaaacaatgcaattgaacccagatcattcagtcagaatccacctgtgctgaagaggcaccagagagagatcactaggactaccctgcagtcagatcaggaagagattgactatgatgataccatctcagtggaaatgaagaaagaggactttgatatctatgatgaagatgagaaccagagtccaaggtctttccagaagaaaaccagacattactttattgctgcagtggagaggctgtgggattatggaatgtcctcaagtccacatgtgctgaggaatagggcacagtctggcagtgtccctcagttcaagaaagtggtcttccaggagtttacagatggcagcttcactcagcctctgtacaggggagaactcaatgagcacctggggctgctgggaccctatatcagagctgaagtggaggataacatcatggtcaccttcaggaatcaggcttcaagaccctacagtttttattctagcctgatcagctatgaagaggaccagaggcagggagctgaacctaggaaaaactttgtgaagccaaatgagaccaaaacatacttttggaaggtccagcaccacatggcaccaaccaaagatgagtttgattgcaaggcatgggcctatttttcagatgtggatctggagaaggatgtccacagtggcctcattgggcctctgctggtgtgccatactaacaccctgaatccagctcatggcaggcaggtgacagtccaggagtttgcactgttctttaccatctttgatgagacaaagtcctggtacttcactgaaaacatggagaggaattgcagagctccttgcaacatccagatggaagaccccaccttcaaggagaactacagatttcatgcaatcaatgggtatatcatggatacactgccaggactggtgatggcccaggaccagaggatcagatggtatctgctcagcatggggtccaatgagaatatccactctatccatttcagtggacatgtgtttacagtcagaaagaaagaagagtataaaatggccctgtacaacctctatccaggagtgtttgaaacagtggagatgctgccaagcaaggctgggatctggagggtggaatgcctcattggggagcacctgcatgcaggaatgtcaaccctgtttctggtctacagtaataagtgccagacacctctgggaatggcaagtggacatatcagggatttccagatcactgctagtggacagtatggacagtgggcaccaaagctggctagactccactattcaggctcaatcaatgcttggtccaccaaagagccattctcatggatcaaggtggacctgctggctcctatgatcatccatggcatcaaaacacagggggcaaggcagaagttctcctcactgtacatctctcagtttatcatcatgtatagcctggatggcaagaaatggcagacctacaggggcaatagcacagggactctgatggtgttctttggcaatgtggacagcagtgggatcaagcacaacatcttcaatcccccaatcattgcaaggtacatcagactgcaccccacccattattcaatcaggagtacactcaggatggaactgatggggtgtgatctcaacagttgctctatgccactgggaatggagtccaaggcaatctcagatgcccagatcactgctagctcctacttcactaatatgtttgctacctggagcccctccaaagcaaggctgcacctccagggaaggagcaatgcatggaggcctcaggtgaacaatcccaaggaatggctgcaggtggatttccagaaaactatgaaggtgactggagtcacaactcagggagtgaaaagtctgctcacttctatgtatgtcaaggagttcctgatctcaagttctcaggatggccaccagtggaccctgttctttcagaatggaaaggtgaaagtcttccagggcaatcaggattcctttacaccagtggtcaactcactggaccctcccctgctcactagatatctgagaatccaccctcagagctgggtgcatcagattgctctcagaatggaagtcctgggctgtgaggcacaggacctgtattga

SEQ ID NO: 127 - DNA, 1386 bp, Artificial Sequence
  recombinant promoter sequence
atgcagagggtgaatatgattatggctgagtcccctgggctgattaccatttgcctgctgggatacctgctgtctgctgagtgtacagtgttcctggaccatgagaatgcaaataagatcctgaacaggcccaaaagatataatagtggaaagctggaggaatttgtgcagggcaacctggagagagaatgcatggaggaaaagtgtagctttgaggaagccagggaggtgtttgaaaatacagagagaaccacagaattctggaagcagtatgtggatggagatcagtgtgagagcaacccctgtctgaatggagggagttgcaaagatgatatcaactcatatgaatgctggtgtccttttggatttgaaggcaaaaattgtgagctggatgtgacctgtaacattaagaatgggaggtgtgagcagttttgtaaaaactctgctgataataaggtggtctgcagttgtacagaagggtatagactggctgagaaccagaagtcctgtgaaccagctgtgcccttcccttgtggaagggtgtctgtctcccagacttcaaaactgaccagagctgagactgtgtttcctgatgtggattatgtcaacagcacagaggctgaaactatcctggacaacattactcagtctacccagagtttcaatgactttaccagagtggtgggaggagaggatgctaaaccaggccagttcccctggcaggtggtcctgaatgggaaggtggatgcattttgtgggggatctattgtgaatgagaaatggattgtcacagctgctcactgtgtggaaactggggtcaagatcacagtggtggctggagagcacaacattgaggaaacagaacatactgagcagaagaggaatgtgatcagaatcattcctcaccataactacaatgcagccatcaacaaatataatcatgacattgccctgctggaactggatgagcctctggtgctgaacagctatgtcacaccaatctgcattgctgacaaggagtacactaacatcttcctgaagtttgggtcaggatatgtgtctggatggggaagagtcttccacaagggcaggtctgcactggtgctgcagtatctgagagtgcctctggtggatagggccacttgtctgctgtctaccaagttcaccatctacaacaatatgttctgtgctggatttcatgagggagggagagactcctgtcagggagattctggaggcccacatgtgacagaggtggaaggcaccagcttcctgacaggcatcatttcctggggggaggaatgtgcaatgaaggggaaatatggaatctacaccaaagtgagcaggtatgtgaactggatcaaggaaaagaccaaactgacatga

SEQ ID NO: 128 - DNA, 252 bp, Artificial Sequence
  recombinant promoter sequence
tgtttgctgcttgcaatgtttgcccattttagggtggacacaggacgctgtggtttctgagccagggggcgactcagatcccagccagtggacttagcccctgtttgctcctccgataactggggtgaccttggttaatattcaccagcagcctcccccgttgcccctctggatccactgcttaaatacggacgaggacagggccctgtctcctcagcttcaggcaccaccactgacctgggacagtgaatc

SEQ ID NO: 129 - DNA, 4882 bp, Artificial Sequence
  recombinant AAV sequence
cctgcaggcagctgcgcgctcgctcgctcactgaggccgcccgggcaaagcccgggcgtcgggcgacctttggtcgcccggcctcagtgagcgagcgagcgcgcagagagggagtggccaactccatcactaggggttcctaccggtgttaatcattaagtcgttaatttttgtggcccttgcgatgtttgctctggttaataatctcaggacaaacagaggttaataattttccagatctctctgagcaatagtataaaaggccagcagcagcctgaccacatctcatcctcgtcgagccaccatgcagatcgaactgtctacctgtttctttctgtgcctgctgcggttttgtttttccgctaccagaagatactacctgggagccgtcgaactgagctgggattacatgcagtctgacctgggagagctgcccgtggacgctagattcccacctagagtccctaagtccttccccttcaacaccagcgtggtctacaagaaaaccctgttcgtggagtttaccgaccacctgttcaacatcgctaagcctagaccaccatggatgggactgctgggaccaaccatccaggccgaggtgtacgacaccgtggtcatcaccctgaaaaacatggcttctcaccccgtgtccctgcatgctgtgggcgtctcctactggaaggccagcgaaggggctgagtatgacgatcagaccagccagcgggaaaaagaggacgataaggtgttccctggcgggtcccatacctacgtgtggcaggtcctgaaggagaatggaccaatggcttccgaccctctgtgcctgacctactcttatctgtcccacgtggacctggtcaaggatctgaacagcggcctgatcggggctctgctggtgtgtcgcgaagggtccctggccaaggagaaaacccagaccctgcataagttcatcctgctgttcgccgtgtttgacgaaggaaaaagctggcactctgagaccaagaactctctgatgcaggacagggatgccgcttccgccagagcttggcccaagatgcacaccgtgaacggctacgtcaataggagcctgcctggactgatcggctgccacagaaagtccgtgtattggcatgtcatcggaatgggcaccacccctgaagtgcacagcatcttcctggaggggcatacctttctggtccgcaaccaccggcaggctagcctggagatctctccaatcaccttcctgaccgcccagaccctgctgatggacctgggacagttcctgctgttttgccacatctccagccaccagcatgatggcatggaggcttacgtgaaagtcgactcctgtcccgaggaacctcagctgaggatgaagaacaatgaggaagccgaagactatgacgatgacctgaccgacagcgagatggatgtggtccgcttcgatgacgataactctccctcctttatccagatccggtccgtggccaagaaacaccctaagacctgggtccattacatcgccgctgaggaagaggactgggattatgctccactggtgctggcccccgacgatagatcctacaaaagccagtatctgaacaatggaccccagaggatcggcagaaagtacaagaaagtgaggttcatggcttataccgatgagacctttaagaccagagaagccatccagcacgagtccgggatcctgggacctctgctgtacggcgaagtgggggacaccctgctgatcatcttcaagaaccaggccagcaggccttacaatatctatccacatggcatcaccgatgtgagacctctgtactcccgccggctgccaaagggcgtgaaacacctgaaggacttcccaatcctgcccggggaaatctttaagtataaatggaccgtcaccgtcgaggatgggcccaccaagagcgaccctaggtgcctgaccagatactattcttccttcgtgaatatggagagagacctggcttccggactgatcggacccctgctgatctgttacaaagagagcgtggatcagcgcggcaaccagatcatgtctgacaagcggaatgtgatcctgttcagcgtctttgacgaaaaccgctcttggtacctgaccgagaacatccagcggttcctgcctaatccagctggagtgcagctggaagatcccgagttccaggcctctaacatcatgcattccatcaatggctacgtgttcgactccctgcagctgagcgtgtgcctgcacgaggtcgcttactggtatatcctgagcatcggagcccagaccgatttcctgtctgtgttcttttccggctacacctttaagcataaaatggtgtatgaggacaccctgaccctgttcccattttccggcgaaaccgtgttcatgagcatggagaatcccgggctgtggatcctgggatgccacaactccgatttcaggaatagagggatgaccgccctgctgaaagtgagctcttgtgacaagaacaccggagactactatgaagatagctacgaggacatctctgcttatctgctgtccaaaaacaatgccatcgagcccaggagcttctctcagaaccctccagtgctgaagcgccaccagcgggagatcaccagaaccaccctgcagagcgatcaggaagagatcgactacgacgataccatctccgtggaaatgaagaaagaggacttcgatatctatgacgaagatgagaaccagtctcccaggtccttccagaagaaaaccagacattactttatcgccgctgtggagcggctgtgggactatggcatgtccagctctcctcacgtgctgagaaatagagctcagtccggaagcgtcccacagttcaagaaagtggtcttccaggagtttaccgacggaagctttacccagccactgtaccgcggcgaactgaacgagcacctggggctgctgggaccctatatccgggctgaagtggaggataacatcatggtcaccttcaggaatcaggccagcagaccctactctttttattccagcctgatctcctacgaagaggaccagagacagggagctgaaccaagaaaaaacttcgtgaagcctaatgagaccaaaacctacttttggaaggtgcagcaccatatggcccctaccaaagacgagttcgattgcaaggcctgggcttattttagcgacgtggatctggagaaggacgtccactccggcctgatcgggccactgctggtgtgtcataccaacaccctgaatccagctcacggaaggcaggtgaccgtccaggaattcgccctgttctttaccatctttgatgagaccaagagctggtacttcaccgaaaacatggagaggaattgcagagccccatgtaacatccagatggaagaccccaccttcaaggagaactacagatttcatgctatcaatgggtatatcatggataccctgccaggactggtcatggctcaggaccagaggatcagatggtacctgctgagcatggggtctaacgagaatatccactccatccatttcagcggacacgtgtttaccgtccgcaagaaagaagagtacaagatggccctgtacaacctgtatcccggcgtgttcgaaaccgtcgagatgctgccttccaaggctgggatctggcgggtggaatgcctgatcggggagcacctgcatgccggaatgtctaccctgttcctggtgtactccaataagtgtcagacccccctggggatggctagcggacatatccgcgacttccagatcaccgcttccggacagtacggacagtgggctcctaagctggctagactgcactattctggctccatcaacgcttggtctaccaaagagcctttctcctggatcaaggtggacctgctggctccaatgatcatccatggcatcaaaacccagggggccaggcagaagttctcttccctgtacatcagccagtttatcatcatgtattctctggatgggaagaaatggcagacctacagaggcaattccaccgggaccctgatggtgttctttggcaacgtcgacagctctgggatcaagcacaacatcttcaatccccctatcatcgcccgctacatccggctgcacccaacccattattccatccgcagcaccctgcggatggagctgatggggtgcgatctgaacagctgttctatgcccctgggaatggagtctaaggccatctccgacgctcagatcaccgcctccagctacttcaccaatatgtttgctacctggtccccaagcaaggctagactgcatctgcagggaagaagcaacgcttggagaccacaggtgaacaatcccaaggagtggctgcaggtcgacttccagaaaaccatgaaggtgaccggagtcaccacccagggcgtgaaaagcctgctgacctctatgtacgtcaaggagttcctgatctcttccagccaggacgggcaccagtggaccctgttctttcagaacggaaaggtgaaagtcttccagggcaatcaggattcctttacccctgtggtcaacagcctggacccacccctgctgaccaggtacctgagaatccacccacagtcctgggtgcatcagatcgctctgaggatggaagtcctgggctgcgaggcccaggacctgtattgagcggccgcaataaaatatctttattttcattacatctgtgtgttggttttttgtgtgcaattgaggaacccctagtgatggagttggccactccctctctgcgcgctcgctcgctcactgaggccgggcgaccaaaggtcgcccgacgcccgggctttgcccgggcggcctcagtgagcgagcgagcgcgcagctgcctgcagg

SEQ ID NO: 130 - DNA, 5018 bp, Artificial Sequence
  recombinant AAV sequence
cctgcaggcagctgcgcgctcgctcgctcactgaggccgcccgggcaaagcccgggcgtcgggcgacctttggtcgcccggcctcagtgagcgagcgagcgcgcagagagggagtggccaactccatcactaggggttcctaccggtgttaatcattaagtcgttaatttttgtggcccttgcgatgtttgctctggttaataatctcaggacaaacagaggttaataattttccagatctctctgagcaatagtataaaaggccagcagcagcctgaccacatctcatcctcgtcgacttaattaaaagaggtaagggtttaagggatggttggttggtggggtattaatgtttaattacctggagcacctgcctgaaatcactttttttcaggttggctcgagccaccatgcagctggaactgtctacctgtgtgtttctgtgtctgctgcctctggggttttctgctatcaggagatactatctgggagctgtggagctgtcctgggactacaggcagtctgagctgctgagagaactgcatgtggataccagattcccagctacagctccaggagctctgcctctgggcccatctgtgctgtacaagaaaacagtctttgtggagtttacagaccagctgttctctgtggccaggccaagaccaccttggatgggactgctgggaccaaccatccaggctgaggtgtatgatacagtggtggtgaccctgaaaaacatggcctcccatcctgtgagcctgcatgctgtgggggtgtccttctggaagtcctctgagggagctgagtatgaagaccatacctcccagagggagaaagaagatgataaggtgctgcctggcaaaagccagacctatgtctggcaggtgctgaaggagaatggaccaactgcttctgacccaccatgcctgacctactcttatctgtcccatgtggatctggtgaaggacctgaattctggactgattggagctctgctggtgtgtagagagggaagcctgaccagagaaagaacccagaacctgcatgagtttgtcctgctgtttgctgtgtttgatgaagggaagagctggcactctgccaggaatgactcctggaccagagctatggatccagctcctgctagagctcagcctgctatgcacacagtcaatggctatgtgaataggtctctgccaggactgattggctgccataagaaatctgtctattggcatgtgattggaatgggcaccagccctgaggtgcattctatcttcctggaaggccacacctttctggtcaggcaccatagacaggcctctctggagatctcccctctgaccttcctgacagctcagacctttctgatggacctggggcagttcctgctgttttgccatatctcttcccaccatcatggaggaatggaggctcatgtcagggtggaatcctgtgctgaggaaccacagctgagaagaaaggctgatgaggaagaggactatgatgataacctgtatgactctgatatggatgtggtgaggctggatggggatgatgtcagccctttcatccagatcaggtctgtggccaagaaacatccaaagacctgggtccactacattgctgctgaagaggaagattgggactatgcccccctggtgctggctcctgatgatagatcctacaaaagccagtatctgaacaatgggccccagaggattggaaggaagtacaagaaagtgaggttcatggcctatacagatgagacctttaagaccagagaggctatccagcatgaatctgggatcctgggacctctgctgtatggagaagtgggggataccctgctgatcatcttcaagaaccaggcctccaggccatacaatatctatccccatggcatcacagatgtgagaccactgtacagcaggagactgcccaagggggtcaaacacctgaaggatttccccatcctgcctggagagatctttaagtataaatggacagtcacagtggaagatgggcctaccaagtctgatccaaggtgcctgaccagatactatagctcttttgtgaacatggagagagacctggcttctggactgattggacccctgctgatctgttacaaagagtctgtggaccagaggggcaaccagatcatgtctgataagagaaatgtcatcctgttctctgtgtttgatgagaacaggagctggtacctgacagagaacatccagaggttcctgccaaatccagctggagtgcagctggaggacccagaatttcaggcttccaacatcatgcatagcatcaatggctatgtgtttgatagcctgcagctgtctgtctgcctgcatgaggtggcctactggtatatcctgtccattggagctcagacagacttcctgtctgtgttctttagtgggtacacctttaagcataaaatggtgtatgaggataccctgaccctgttccccttttctggggagacagtgttcatgtccatggaaaaccctggcctgtggatcctggggtgccacaactctgacttcaggaatagaggaatgacagccctgctgaaagtgtccagctgtgataagaatacaggggattactatgaggactcttatgaagatatctctgcttatctgctgagcaagaacaatgccattgagcccaggtcttttgctcagaactccagacctccatctgcttctgctcctaagccacctgtgctgagaagacatcagagggacatctccctgcctaccttccagccagaggaagataaaatggactatgatgatatcttcagcacagagaccaagggggaagattttgacatctatggagaggatgaaaaccaggatccaagatccttccagaagagaaccagacactactttattgctgctgtggagcagctgtgggactatgggatgtctgaaagcccaagggccctgaggaacagagctcagaatggagaggtgcccagattcaagaaagtggtgttcagagagtttgctgatggcagctttacccagccatcttacaggggggagctgaacaagcatctggggctgctgggaccctatatcagagctgaggtggaagataacatcatggtgaccttcaagaatcaggcttctaggccctactccttttattcttccctgatctcctaccctgatgatcaggagcagggagctgaacctaggcacaactttgtgcagccaaatgagaccagaacctacttttggaaggtgcagcatcacatggctcccacagaggatgaatttgactgcaaagcttgggcctatttttctgatgtggacctggagaaggatgtgcattctggcctgattgggcctctgctgatctgtagggccaacaccctgaatgctgctcatggaagacaggtcacagtgcaggagtttgctctgttctttaccatctttgatgaaaccaagagctggtacttcacagagaatgtggaaaggaattgcagagccccctgtcatctgcagatggaggaccctaccctgaaggaaaactacaggttccatgccatcaatggatatgtcatggataccctgcctggcctggtcatggctcagaaccagaggatcagatggtacctgctgtctatgggatccaatgagaatatccatagcatccacttctctggccatgtcttttctgtgaggaagaaagaggaatacaaaatggctgtgtacaatctgtatcctggggtctttgagacagtggaaatgctgccaagcaaagtgggaatctggagaattgagtgcctgattggggaacacctgcaggctgggatgagcaccaccttcctggtgtactctaagaaatgtcagaccccactggggatggcctctggacatatcagggacttccagatcacagcttctggacagtatggacagtgggctccaaagctggctagactgcactattctggctccatcaatgcctggtctaccaaagagccattctcctggatcaaggtggacctgctggcccccatgatcatccatggaatcaaaacccagggagctaggcagaagttcagctctctgtacatctcccagtttatcatcatgtatagcctggatgggaagaaatggcagacctacagaggcaattccactgggaccctgatggtcttctttggaaatgtggattcctctggcatcaagcacaacatcttcaatccacccatcattgccaggtacatcaggctgcatcctacccactatagcatcaggtctaccctgagaatggagctgatgggatgtgacctgaacagctgttctatgccactgggcatggagtccaaggctatctctgatgcccagatcacagcttcttcctacttcaccaatatgtttgctacctggtccccaagcaaggctagactgcacctgcagggaagatccaatgcttggagaccccaggtgaacaatcctaaggagtggctgcaggtggacttccagaaaaccatgaaggtcacaggggtgaccacccagggagtgaaatctctgctgacctccatgtatgtcaaggagttcctgatcagctcttcccaggatggccaccagtggaccctgttctttcagaatggcaaggtcaaagtgttccaggggaatcaggactcttttaccccagtggtgaactccctggatcctccactgctgaccaggtacctgagaatccatcctcagagctgggtgcaccagattgctctgagaatggaggtcctgggatgtgaagctcaggacctgtattgagcggccgcaataaaatatctttattttcattacatctgtgtgttggttttttgtgtgcaattgaggaacccctagtgatggagttggccactccctctctgcgcgctcgctcgctcactgaggccgggcgaccaaaggtcgcccgacgcccgggctttgcccgggcggcctcagtgagcgagcgagcgcgcagctgcctgcagg

SEQ ID NO: 131 - DNA, 137 bp, Artificial Sequence
  recombinant promoter sequence
gttaatttttaaaaagcagtcaaaagtccaagtggcccttgcgagcatttactctctctgtttgctctggttaataatctcaggagcacaaacagaggttaataattttccagatctctctgagcaatagtataaaa